European Patent Specification EP 3 517 544 B1, published January 8, 2025. Title: Insulin analogs with reduced affinity to insulin receptor and use thereof. Applicant: HANMI PHARM. CO., LTD. Sanofi-Aventis Deutschland GmbH. The sequence listing filed with the application follows.

SEQUENCE LISTING (56 sequences)

SEQ ID NO: 1 - DNA, 34 bp, Artificial Sequence
  Primer
cagcatctgctccctccatcagctggagaactac

SEQ ID NO: 2 - DNA, 34 bp, Artificial Sequence
  Primer
gtagttctccagctgatggagggagcagatgctg

SEQ ID NO: 3 - DNA, 34 bp, Artificial Sequence
  Primer
cagcatctgctccctcaagcagctggagaactac

SEQ ID NO: 4 - DNA, 34 bp, Artificial Sequence
  Primer
gtagttctccagctgcttgagggagcagatgctg

SEQ ID NO: 5 - DNA, 34 bp, Artificial Sequence
  Primer
ctaccagctggagaacgagtgcaactgaggatcc

SEQ ID NO: 6 - DNA, 34 bp, Artificial Sequence
  Primer
ggatcctcagttgcactcgttctccagctggtag

SEQ ID NO: 7 - DNA, 34 bp, Artificial Sequence
  Primer
ctaccagctggagaactcctgcaactgaggatcc

SEQ ID NO: 8 - DNA, 34 bp, Artificial Sequence
  Primer
ggatcctcagttgcaggagttctccagctggtag

SEQ ID NO: 9 - DNA, 34 bp, Artificial Sequence
  Primer
ctaccagctggagaacacctgcaactgaggatcc

SEQ ID NO: 10 - DNA, 34 bp, Artificial Sequence
  Primer
ggatcctcagttgcaggtgttctccagctggtag

SEQ ID NO: 11 - DNA, 34 bp, Artificial Sequence
  Primer
ctggtggaagctctcgagctagtgtgcggggaac

SEQ ID NO: 12 - DNA, 34 bp, Artificial Sequence
  Primer
gttccccgcacactagctcgagagcttccaccag

SEQ ID NO: 13 - DNA, 34 bp, Artificial Sequence
  Primer
ctggtggaagctctctccctagtgtgcggggaac

SEQ ID NO: 14 - DNA, 34 bp, Artificial Sequence
  Primer
gttccccgcacactagggagagagcttccaccag

SEQ ID NO: 15 - DNA, 34 bp, Artificial Sequence
  Primer
ctggtggaagctctcaccctagtgtgcggggaac

SEQ ID NO: 16 - DNA, 34 bp, Artificial Sequence
  Primer
gttccccgcacactagggtgagagcttccaccag

SEQ ID NO: 17 - DNA, 34 bp, Artificial Sequence
  Primer
cagcatctgctccctcgcccagctggagaactac

SEQ ID NO: 18 - DNA, 34 bp, Artificial Sequence
  Primer
gtagttctccagctgggcgagggagcagatgctg

SEQ ID NO: 19 - DNA, 34 bp, Artificial Sequence
  Primer
cagcatctgctccctcgaccagctggagaactac

SEQ ID NO: 20 - DNA, 34 bp, Artificial Sequence
  Primer
gtagttctccagctggtcgagggagcagatgctg

SEQ ID NO: 21 - DNA, 34 bp, Artificial Sequence
  Primer
ctggtggaagctctcgacctagtgtgcggggaac

SEQ ID NO: 22 - DNA, 34 bp, Artificial Sequence
  Primer
gttccccgcacactaggtcgagagcttccaccag

SEQ ID NO: 23 - DNA, 33 bp, Artificial Sequence
  Primer
ggggaacgaggcttcgactacacacccaagacc

SEQ ID NO: 24 - DNA, 33 bp, Artificial Sequence
  Primer
ggtcttgggtgtgtagtcgaagcctcgttcccc

SEQ ID NO: 25 - DNA, 33 bp, Artificial Sequence
  Primer
ggggaacgaggcttcgagtacacacccaagacc

SEQ ID NO: 26 - DNA, 33 bp, Artificial Sequence
  Primer
ggtcttgggtgtgtactcgaagcctcgttcccc

SEQ ID NO: 27 - DNA, 258 bp, Artificial Sequence
  Analog 1
ttcgttaaccaacacttgtgtggctcacacctggtggaagctctctacctagtgtgcggggaacgaggcttcttctacacacccaagacccgccgggaggcagaggacctgcaggtggggcaggtggagctgggcgggggccctggtgcaggcagcctgcagcccttggccctggaggggtccctgcagaagcgtggcattgtggaacaatgctgtaccagcatctgctccctccatcagctggagaactactgcaac

SEQ ID NO: 28 - protein, 86 aa, Artificial Sequence
  Analog 1
FVNQHLCGSHLVEALYLVCGERGFFYTPKTRREAEDLQVGQVELGGGPGAGSLQPLALEGSLQKRGIVEQCCTSICSLHQLENYCN

SEQ ID NO: 29 - DNA, 258 bp, Artificial Sequence
  Analog 2
ttcgttaaccaacacttgtgtggctcacacctggtggaagctctctacctagtgtgcggggaacgaggcttcttctacacacccaagacccgccgggaggcagaggacctgcaggtggggcaggtggagctgggcgggggccctggtgcaggcagcctgcagcccttggccctggaggggtccctgcagaagcgtggcattgtggaacaatgctgtaccagcatctgctccctcaagcagctggagaactactgcaac

SEQ ID NO: 30 - protein, 86 aa, Artificial Sequence
  Analog 2
FVNQHLCGSHLVEALYLVCGERGFFYTPKTRREAEDLQVGQVELGGGPGAGSLQPLALEGSLQKRGIVEQCCTSICSLKQLENYCN

SEQ ID NO: 31 - DNA, 258 bp, Artificial Sequence
  Analog 3
ttcgttaaccaacacttgtgtggctcacacctggtggaagctctctacctagtgtgcggggaacgaggcttcttctacacacccaagacccgccgggaggcagaggacctgcaggtggggcaggtggagctgggcgggggccctggtgcaggcagcctgcagcccttggccctggaggggtccctgcagaagcgtggcattgtggaacaatgctgtaccagcatctgctccctctaccagctggagaacgagtgcaac

SEQ ID NO: 32 - protein, 86 aa, Artificial Sequence
  Analog 3
FVNQHLCGSHLVEALYLVCGERGFFYTPKTRREAEDLQVGQVELGGGPGAGSLQPLALEGSLQKRGIVEQCCTSICSLYQLENECN

SEQ ID NO: 33 - DNA, 258 bp, Artificial Sequence
  Analog 4
ttcgttaaccaacacttgtgtggctcacacctggtggaagctctctacctagtgtgcggggaacgaggcttcttctacacacccaagacccgccgggaggcagaggacctgcaggtggggcaggtggagctgggcgggggccctggtgcaggcagcctgcagcccttggccctggaggggtccctgcagaagcgtggcattgtggaacaatgctgtaccagcatctgctccctctaccagctggagaactcctgcaac

SEQ ID NO: 34 - protein, 86 aa, Artificial Sequence
  Analog 4
FVNQHLCGSHLVEALYLVCGERGFFYTPKTRREAEDLQVGQVELGGGPGAGSLQPLALEGSLQKRGIVEQCCTSICSLYQLENSCN

SEQ ID NO: 35 - DNA, 258 bp, Artificial Sequence
  Analog 5
ttcgttaaccaacacttgtgtggctcacacctggtggaagctctctacctagtgtgcggggaacgaggcttcttctacacacccaagacccgccgggaggcagaggacctgcaggtggggcaggtggagctgggcgggggccctggtgcaggcagcctgcagcccttggccctggaggggtccctgcagaagcgtggcattgtggaacaatgctgtaccagcatctgctccctctaccagctggagaacacctgcaac

SEQ ID NO: 36 - protein, 86 aa, Artificial Sequence
  Analog 5
FVNQHLCGSHLVEALYLVCGERGFFYTPKTRREAEDLQVGQVELGGGPGAGSLQPLALEGSLQKRGIVEQCCTSICSLYQLENTCN

SEQ ID NO: 37 - DNA, 258 bp, Artificial Sequence
  Analog 6
ttcgttaaccaacacttgtgtggctcacacctggtggaagctctcgagctagtgtgcggggaacgaggcttcttctacacacccaagacccgccgggaggcagaggacctgcaggtggggcaggtggagctgggcgggggccctggtgcaggcagcctgcagcccttggccctggaggggtccctgcagaagcgtggcattgtggaacaatgctgtaccagcatctgctccctctaccagctggagaactactgcaac

SEQ ID NO: 38 - protein, 86 aa, Artificial Sequence
  Analog 6
FVNQHLCGSHLVEALELVCGERGFFYTPKTRREAEDLQVGQVELGGGPGAGSLQPLALEGSLQKRGIVEQCCTSICSLYQLENYCN

SEQ ID NO: 39 - DNA, 258 bp, Artificial Sequence
  Analog 7
ttcgttaaccaacacttgtgtggctcacacctggtggaagctctctccctagtgtgcggggaacgaggcttcttctacacacccaagacccgccgggaggcagaggacctgcaggtggggcaggtggagctgggcgggggccctggtgcaggcagcctgcagcccttggccctggaggggtccctgcagaagcgtggcattgtggaacaatgctgtaccagcatctgctccctctaccagctggagaactactgcaac

SEQ ID NO: 40 - protein, 86 aa, Artificial Sequence
  Analog 7
FVNQHLCGSHLVEALSLVCGERGFFYTPKTRREAEDLQVGQVELGGGPGAGSLQPLALEGSLQKRGIVEQCCTSICSLYQLENYCN

SEQ ID NO: 41 - DNA, 258 bp, Artificial Sequence
  Analog 8
ttcgttaaccaacacttgtgtggctcacacctggtggaagctctcaccctagtgtgcggggaacgaggcttcttctacacacccaagacccgccgggaggcagaggacctgcaggtggggcaggtggagctgggcgggggccctggtgcaggcagcctgcagcccttggccctggaggggtccctgcagaagcgtggcattgtggaacaatgctgtaccagcatctgctccctctaccagctggagaactactgcaac

SEQ ID NO: 42 - protein, 86 aa, Artificial Sequence
  Analog 8
FVNQHLCGSHLVEALTLVCGERGFFYTPKTRREAEDLQVGQVELGGGPGAGSLQPLALEGSLQKRGIVEQCCTSICSLYQLENYCN

SEQ ID NO: 43 - DNA, 258 bp, Artificial Sequence
  Analog 9
ttcgttaaccaacacttgtgtggctcacacctggtggaagctctctacctagtgtgcggggaacgaggcttcttctacacacccaagacccgccgggaggcagaggacctgcaggtggggcaggtggagctgggcgggggccctggtgcaggcagcctgcagcccttggccctggaggggtccctgcagaagcgtggcattgtggaacaatgctgtaccagcatctgctccctcgcccagctggagaactactgcaac

SEQ ID NO: 44 - protein, 86 aa, Artificial Sequence
  Analog 9
FVNQHLCGSHLVEALYLVCGERGFFYTPKTRREAEDLQVGQVELGGGPGAGSLQPLALEGSLQKRGIVEQCCTSICSLAQLENYCN

SEQ ID NO: 45 - DNA, 258 bp, Artificial Sequence
  Analog 10
ttcgttaaccaacacttgtgtggctcacacctggtggaagctctctacctagtgtgcggggaacgaggcttcttctacacacccaagacccgccgggaggcagaggacctgcaggtggggcaggtggagctgggcgggggccctggtgcaggcagcctgcagcccttggccctggaggggtccctgcagaagcgtggcattgtggaacaatgctgtaccagcatctgctccctcgaccagctggagaactactgcaac

SEQ ID NO: 46 - protein, 86 aa, Artificial Sequence
  Analog 10
FVNQHLCGSHLVEALYLVCGERGFFYTPKTRREAEDLQVGQVELGGGPGAGSLQPLALEGSLQKRGIVEQCCTSICSLDQLENYCN

SEQ ID NO: 47 - DNA, 258 bp, Artificial Sequence
  Analog 11
ttcgttaaccaacacttgtgtggctcacacctggtggaagctctcgacctagtgtgcggggaacgaggcttcttctacacacccaagacccgccgggaggcagaggacctgcaggtggggcaggtggagctgggcgggggccctggtgcaggcagcctgcagcccttggccctggaggggtccctgcagaagcgtggcattgtggaacaatgctgtaccagcatctgctccctctaccagctggagaactactgcaac

SEQ ID NO: 48 - protein, 86 aa, Artificial Sequence
  Analog 11
FVNQHLCGSHLVEALDLVCGERGFFYTPKTRREAEDLQVGQVELGGGPGAGSLQPLALEGSLQKRGIVEQCCTSICSLYQLENYCN

SEQ ID NO: 49 - DNA, 258 bp, Artificial Sequence
  Analog 12
ttcgttaaccaacacttgtgtggctcacacctggtggaagctctctacctagtgtgcggggaacgaggcttcgactacacacccaagacccgccgggaggcagaggacctgcaggtggggcaggtggagctgggcgggggccctggtgcaggcagcctgcagcccttggccctggaggggtccctgcagaagcgtggcattgtggaacaatgctgtaccagcatctgctccctctaccagctggagaactactgcaac

SEQ ID NO: 50 - protein, 86 aa, Artificial Sequence
  Analog 12
FVNQHLCGSHLVEALYLVCGERGFDYTPKTRREAEDLQVGQVELGGGPGAGSLQPLALEGSLQKRGIVEQCCTSICSLYQLENYCN

SEQ ID NO: 51 - DNA, 258 bp, Artificial Sequence
  Analog 13
ttcgttaaccaacacttgtgtggctcacacctggtggaagctctctacctagtgtgcggggaacgaggcttcgagtacacacccaagacccgccgggaggcagaggacctgcaggtggggcaggtggagctgggcgggggccctggtgcaggcagcctgcagcccttggccctggaggggtccctgcagaagcgtggcattgtggaacaatgctgtaccagcatctgctccctctaccagctggagaactactgcaac

SEQ ID NO: 52 - protein, 86 aa, Artificial Sequence
  Analog 13
FVNQHLCGSHLVEALYLVCGERGFEYTPKTRREAEDLQVGQVELGGGPGAGSLQPLALEGSLQKRGIVEQCCTSICSLYQLENYCN

SEQ ID NO: 53 - protein, 21 aa, Homo sapiens
GIVEQCCTSICSLYQLENYCN

SEQ ID NO: 54 - protein, 30 aa, Homo sapiens
FVNQHLCGSHLVEALYLVCGERGFFYTPKT

SEQ ID NO: 55 - protein, 21 aa, Artificial Sequence
  Insulin analog, A-chain
  MISC_FEATURE (1): Xaa is alanine, glycine, glutamine, histidine, glutamic acid, or asparagine
  MISC_FEATURE (5): Xaa is alanine, glutamic acid, glutamine, histidine, or asparagine
  MISC_FEATURE (12): Xaa is alanine, serine, glutamine, glutamic acid, histidine, or asparagine
  MISC_FEATURE (14): Xaa is tyrosine, histidine, lysine, alanine, or aspartic acid
  MISC_FEATURE (16): Xaa is alanine, leucine, tyrosine, histidine, glutamic acid, or asparagine
  MISC_FEATURE (19): Xaa is tyrosine, glutamic acid, serine, or threonine
  MISC_FEATURE (21): Xaa is asparagine, glycine, histidine, or alanine
XIVEXCCTSICXLXQXENXCX

SEQ ID NO: 56 - protein, 30 aa, Artificial Sequence
  Insulin analog, B-chain
  MISC_FEATURE (16): Xaa is tyrosine, glutamic acid, serine, threonine, or aspartic acid
  MISC_FEATURE (25): Xaa is phenylalanine, aspartic acid, or glutamic acid
  MISC_FEATURE (27): Xaa is threonine, or is absent
  MISC_FEATURE (28): Xaa is proline, glutamic acid, or aspartic acid, or is absent
FVNQHLCGSHLVEALXLVCGERGFXYXXKT